European Patent Application EP 4 174 168 A1, published May 3, 2023. Title: BACILLUS VELEZENSIS STRAIN BRED THROUGH ULTRASOUND-ASSISTED ADAPTIVE EVOLUTION, AND USE THEREOF. Applicant: Jiangsu University. The sequence listing filed with the application follows.

SEQUENCE LISTING (4 sequences)

SEQ ID NO: 1 - DNA, 20 bp, Artificial Sequence
agagtttgatcctggctcag

SEQ ID NO: 2 - DNA, 22 bp, Artificial Sequence
tacggytaccttgttacgactt

SEQ ID NO: 3 - DNA, 1542 bp, Bacillus velezensis
agagtttgatcctggctcaggacgaacgctggcggcgtgcctaatacatgcaagtcgagcggacagatgggagcttgctccctgatgttagcggcggacgggtgagtaacacgtgggtaacctgcctgtaagactgggataactccgggaaaccggggctaataccggatgcttgtttgaaccgcatggttcagacataaaaggtggcttcggctaccacttacagatggacccgcggcgcattagctagttggtgaggtaacggctcaccaaggcaacgatgcgtagccgacctgagagggtgatcggccacactgggactgagacacggcccagactcctacgggaggcagcagtagggaatcttccgcaatggacgaaagtctgacggagcaacgccgcgtgagtgatgaaggttttcggatcgtaaagctctgttgttagggaagaacaagtgccgttcaaatagggcggcaccttgacggtacctaaccagaaagccacggctaactacgtgccagcagccgcggtaatacgtaggtggcaagcgttgtccggaattattgggcgtaaagggctcgcaggcggtttcttaagtctgatgtgaaagcccccggctcaaccggggagggtcattggaaactggggaacttgagtgcagaagaggagagtggaattccacgtgtagcggtgaaatgcgtagagatgtggaggaacaccagcggcgaaggcgactctctggtctgtaactgacgctgaggagcgaaagcgtggggagcgaacaggattagataccctggtagtccacgccgtaaacgatgagtgctaagtgttagggggtttccgccccttagtgctgcagctaacgcattaagcactccgcctggggagtacggtcgcaagactgaaactcaaaggaattgacgggggcccgcacaagcggtggagcatgtggtttaattcgaagcaacgcgaagaaccttaccaggtcttgacatcctctgacaatcctagagataggacgtccccttcgggggcagagtgacaggtggtgcatggttgtcgtcagctcgtgtcgtgagatgttgggttaagtcccgcaacgagcgcaacccttgatcttagttgccagcattcagttgggcactctaaggtgactgccggtgacaaaccggaggaaggtggggatgacgtcaaatcatcatgccccttatggcctgggctacacacgtgctacaatgggcagaacaaagggcagcgaaaccgcgaggttaagccaatcccacaaatctgttctcagttcggatcgcagtctgcaactcgactgcgtgaagctggaatcgctagtaatcgcggatcagcatgccgcggtgaatacgttcccgggccttgtacacaccgcccgtcacaccacgagagtttgtaacacccgaagtcggtgaggtaaccttttaggagccagccgccgaaggtgggacagatgattggggtgaagtcgtaacaaggtagccgtatcggaaggtgcggctggatcacctcctt

SEQ ID NO: 4 - DNA, 1542 bp, Bacillus velezensis; identical to SEQ ID NO: 3